European Patent Specification EP 3 838 286 B1, published October 15, 2025. Title: ANTIMICROBIAL PEPTIDE FROM POLISTES GALLICUS VENOM AND ITS ANALOGS. Applicant: LATOXAN Aix-Marseille-Université (AMU) Centre National de la Recherche Scientifique (CNRS) Mabrouk, Kamel Marseca, Marc De Pomyers, Harold Gigmes, Didier. The sequence listing filed with the application follows.

SEQUENCE LISTING (28 sequences)

SEQ ID NO: 1 - protein, 12 aa, Artificial Sequence
  Consensus sequence for Polistes gallicus peptides
  VARIANT (3)..(3): X=S, K, W or absent
  VARIANT (4)..(4): X=A, L or absent
  VARIANT (5)..(5): X=I or W
  VARIANT (6)..(6): X=L or K
  VARIANT (7)..(7): X=G or K
  VARIANT (10)..(10): X=K or R
ILXXXXXLLXNL

SEQ ID NO: 2 - protein, 12 aa, Artificial Sequence
  Gallicus-CP I1L12
ILSAILGLLKNL

SEQ ID NO: 3 - protein, 12 aa, Artificial Sequence
  L12I1
LNKLLGLIASLI

SEQ ID NO: 4 - protein, 9 aa, Artificial Sequence
  I1L9
ILSAILGLL

SEQ ID NO: 5 - protein, 10 aa, Artificial Sequence
  I1K10
ILSAILGLLK

SEQ ID NO: 6 - protein, 10 aa, Artificial Sequence
  K10I1
KLLGLIASLI

SEQ ID NO: 7 - protein, 9 aa, Artificial Sequence
  L2K10
LSAILGLLK

SEQ ID NO: 8 - protein, 8 aa, Artificial Sequence
  L2L9
LSAILGLL

SEQ ID NO: 9 - protein, 5 aa, Artificial Sequence
  L8L12
LLKNL

SEQ ID NO: 10 - protein, 7 aa, Artificial Sequence
  I6L12
LGLLKNL

SEQ ID NO: 11 - protein, 10 aa, Artificial Sequence
  S3L12
SAILGLLKNL

SEQ ID NO: 12 - protein, 7 aa, Artificial Sequence
  S3L9
SAILGLL

SEQ ID NO: 13 - protein, 12 aa, Artificial Sequence
  (i1l12)enantio
  VARIANT (1)..(1): D-isoleucine
  VARIANT (2)..(2): D-leucine
  VARIANT (3)..(3): D-serine
  VARIANT (4)..(4): D-alanine
  VARIANT (5)..(5): D-isoleucine
  VARIANT (6)..(6): D-leucine
  VARIANT (7)..(7): D-glycine
  VARIANT (8)..(8): D-leucine
  VARIANT (9)..(9): D-leucine
  VARIANT (10)..(10): D-lysine
  VARIANT (11)..(11): D-asparagine
  VARIANT (12)..(12): D-leucine
XXXXXXXXXXXX

SEQ ID NO: 14 - protein, 8 aa, Artificial Sequence
  K1I8
KLLGLILI

SEQ ID NO: 15 - protein, 11 aa, Artificial Sequence
  LTX-gallicune-1 (I1N11)
ILKAIKKLLKN

SEQ ID NO: 16 - protein, 11 aa, Artificial Sequence
  LTX-gallicune-1(i1D-n11D)
  variant (1)..(1): D-isoleucine
  variant (11)..(11): D-asparagine
XLKAIKKLLKX

SEQ ID NO: 17 - protein, 11 aa, Artificial Sequence
  LTX-D (gallicune-1)
  VARIANT (1)..(1): D-isoleucine
  VARIANT (2)..(2): D-leucine
  VARIANT (3)..(3): D-lysine
  VARIANT (4)..(4): D-alanine
  VARIANT (5)..(5): D-isoleucine
  VARIANT (6)..(6): D-lysine
  VARIANT (7)..(7): D-lysine
  VARIANT (8)..(8): D-leucine
  VARIANT (9)..(9): D-leucine
  VARIANT (10)..(10): D-lysine
  VARIANT (11)..(11): D-asparagine
XXXXXXXXXXX

SEQ ID NO: 18 - protein, 9 aa, Artificial Sequence
  I1L9*
ILKAIKKLL

SEQ ID NO: 19 - protein, 7 aa, Artificial Sequence
  I1K7*
ILKAIKK

SEQ ID NO: 20 - protein, 8 aa, Artificial Sequence
  L2L9*
LKAIKKLL

SEQ ID NO: 21 - protein, 9 aa, Artificial Sequence
  L2k10*
  VARIANT (9)..(9): D-lysine
LKAIKKLLX

SEQ ID NO: 22 - protein, 9 aa, Artificial Sequence
  K3N11
KAIKKLLKN

SEQ ID NO: 23 - protein, 10 aa, Artificial Sequence
  AcI1N10*
  MOD_RES (1)..(1): ACETYLATION
IKAIKKLLKN

SEQ ID NO: 24 - protein, 10 aa, Artificial Sequence
  I1K10*
ILKAIKKLLK

SEQ ID NO: 25 - protein, 10 aa, Artificial Sequence
  i1K10*
  VARIANT (1)..(1): D-isoleucine
  VARIANT (10)..(10): D-lysine
XLKAIKKLLX

SEQ ID NO: 26 - protein, 10 aa, Artificial Sequence
  (i1k10*) enantio
  VARIANT (1)..(1): D-isoleucine
  VARIANT (2)..(2): D-leucine
  VARIANT (3)..(3): D-lysine
  VARIANT (4)..(4): D-alanine
  VARIANT (5)..(5): D-isoleucine
  VARIANT (6)..(6): D-lysine
  VARIANT (7)..(7): D-lysine
  VARIANT (8)..(8): D-leucine
  VARIANT (9)..(9): D-leucine
  VARIANT (10)..(10): D-lysine
XXXXXXXXXX

SEQ ID NO: 27 - protein, 8 aa, Artificial Sequence
  LTX-gallicune-2 (R1W8)
RLLGLWLW

SEQ ID NO: 28 - protein, 8 aa, Artificial Sequence
  LTX-gallicune-2 (r1W8)
  variant (1)..(1): D-arginine
XLLGLWLW